European Patent Specification EP 3 737 399 B1, published July 26, 2023. Title: ATF5 PEPTIDE VARIANTS AND USES THEREOF. Applicant: SAPIENCE THERAPEUTICS, INC. The sequence listing filed with the application follows.

SEQUENCE LISTING (87 sequences)

SEQ ID NO: 1 - protein, 76 aa, Artificial Sequence
  Description of Artificial Sequence: Synthetic polypeptide
LEQRAEELARENEELLEKEAEELEQENAELEGECQGLEARNRELRERAESVEREIQYVKDLLIEVYKARSQRTRSA

SEQ ID NO: 2 - protein, 67 aa, Artificial Sequence
  Description of Artificial Sequence: Synthetic polypeptide
RQIKIWFQNRRMKWKKLEQRAEELARENEELLEKEAEELEQENAELEGECQGLEARNRELRERAESV

SEQ ID NO: 3 - protein, 38 aa, Artificial Sequence
  Description of Artificial Sequence: Synthetic polypeptide
RQIKIWFQNRRMKWKKLEGECQGLEARNRELKERAESV

SEQ ID NO: 4 - protein, 38 aa, Artificial Sequence
  Description of Artificial Sequence: Synthetic polypeptide
RQIKIWFQNRRMKWKKLEGEGQGLEARNRELKERAESV

SEQ ID NO: 5 - protein, 38 aa, Artificial Sequence
  Description of Artificial Sequence: Synthetic polypeptide
RQIKIWFQNRRMKWKKLEGEAQGLEARNRELKERAESV

SEQ ID NO: 6 - protein, 38 aa, Artificial Sequence
  Description of Artificial Sequence: Synthetic polypeptide
RQIKIWFQNRRMKWKKLEGECQGLEARNRELKERAEAV

SEQ ID NO: 7 - protein, 38 aa, Artificial Sequence
  Description of Artificial Sequence: Synthetic polypeptide
RQIKIWFQNRRMKWKKLEGECQGLEARLRELKERAESV

SEQ ID NO: 8 - protein, 38 aa, Artificial Sequence
  Description of Artificial Sequence: Synthetic polypeptide
RQIKIWFQNRRMKWKKLEGECAGLEARNRELKERAESV

SEQ ID NO: 9 - protein, 38 aa, Artificial Sequence
  Description of Artificial Sequence: Synthetic polypeptide
RQIKIWFQNRRMKWKKLEGRCQGLRAENRELEERAESV

SEQ ID NO: 10 - protein, 38 aa, Artificial Sequence
  Description of Artificial Sequence: Synthetic polypeptide
RQIKIWFQNRRMKWKKLEGRCQGLRAELRELEERAEAV

SEQ ID NO: 11 - protein, 38 aa, Artificial Sequence
  Description of Artificial Sequence: Synthetic polypeptide
RQIKIWFQNRRMKWKKLEGRAQGLRAELRELEERAEAV

SEQ ID NO: 12 - protein, 38 aa, Artificial Sequence
  Description of Artificial Sequence: Synthetic polypeptide
RQIKIWFQNRRMKWKKLEGRAAGLRAELRELEERAEAV

SEQ ID NO: 13 - protein, 38 aa, Artificial Sequence
  Description of Artificial Sequence: Synthetic polypeptide
  MOD_RES (1)..(38): D-amino acid
VAEAREELERLEARLGQARGELKKWKMRRNQFWIKIQR

SEQ ID NO: 14 - protein, 38 aa, Artificial Sequence
  Description of Artificial Sequence: Synthetic polypeptide
  MOD_RES (1)..(38): D-amino acid
VAEAREELERLEARLGQARGELKKWKMRRNQFWLKLQR

SEQ ID NO: 15 - protein, 7 aa, Artificial Sequence
  Description of Artificial Sequence: Synthetic peptide
FKKFRKF

SEQ ID NO: 16 - protein, 23 aa, Artificial Sequence
  Description of Artificial Sequence: Synthetic peptide
LIRLWSHLIHIWFQNRRLKWKKK

SEQ ID NO: 17 - protein, 27 aa, Artificial Sequence
  Description of Artificial Sequence: Synthetic peptide
GALFLGWLGAAGSTMGAWSQPKKKRKV

SEQ ID NO: 18 - protein, 16 aa, Artificial Sequence
  Description of Artificial Sequence: Synthetic peptide
AAVALLPAVLLALLAP

SEQ ID NO: 19 - protein, 8 aa, Artificial Sequence
  Description of Artificial Sequence: Synthetic peptide
ERKKRRRE

SEQ ID NO: 20 - protein, 22 aa, Artificial Sequence
  Description of Artificial Sequence: Synthetic peptide
LGTYTQDFNKTFPQTAIGVGAP

SEQ ID NO: 21 - protein, 18 aa, Artificial Sequence
  Description of Artificial Sequence: Synthetic peptide
KLALKLALKALKAALKLA

SEQ ID NO: 22 - protein, 27 aa, Artificial Sequence
  Description of Artificial Sequence: Synthetic peptide
GLAFLGFLGAAGSTMGAWSQPKKKRKV

SEQ ID NO: 23 - protein, 10 aa, Artificial Sequence
  Description of Artificial Sequence: Synthetic peptide
VQRKRQKLMP

SEQ ID NO: 24 - protein, 8 aa, Artificial Sequence
  Description of Artificial Sequence: Synthetic peptide
GRKRKKRT

SEQ ID NO: 25 - protein, 16 aa, Artificial Sequence
  Description of Artificial Sequence: Synthetic peptide
RQIKIWFQNRRMKWKK

SEQ ID NO: 26 - protein, 16 aa, Artificial Sequence
  Description of Artificial Sequence: Synthetic peptide
RQLKLWFQNRRMKWKK

SEQ ID NO: 27 - protein, 16 aa, Artificial Sequence
  Description of Artificial Sequence: Synthetic peptide
REIKIWFQNRRMKWKK

SEQ ID NO: 28 - protein, 20 aa, Artificial Sequence
  Description of Artificial Sequence: Synthetic peptide
KETWWETWWTEWSQPKKRKV

SEQ ID NO: 29 - protein, 16 aa, Artificial Sequence
  Description of Artificial Sequence: Synthetic peptide
PVIRVWFQNKRCKDKK

SEQ ID NO: 30 - protein, 12 aa, Artificial Sequence
  Description of Artificial Sequence: Synthetic peptide
  MISC_FEATURE (7)..(12): This region may encompass 1-6 residues
RRRRRRRRRRRR

SEQ ID NO: 31 - protein, 16 aa, Artificial Sequence
  Description of Artificial Sequence: Synthetic peptide
LLIILRRRIRKQAHAH

SEQ ID NO: 32 - protein, 16 aa, Artificial Sequence
  Description of Artificial Sequence: Synthetic peptide
RRLRRLLRRLLRRLRR

SEQ ID NO: 33 - protein, 12 aa, Artificial Sequence
  Description of Artificial Sequence: Synthetic peptide
RVGRRRRRRRRR

SEQ ID NO: 34 - protein, 9 aa, Artificial Sequence
  Description of Artificial Sequence: Synthetic peptide
RRWWRRWRR

SEQ ID NO: 35 - protein, 27 aa, Artificial Sequence
  Description of Artificial Sequence: Synthetic peptide
MGLGLHLLVLAAALQGAWSQPKKKRKV

SEQ ID NO: 36 - protein, 7 aa, Artificial Sequence
  Description of Artificial Sequence: Synthetic peptide
PKKKRKV

SEQ ID NO: 37 - protein, 18 aa, Artificial Sequence
  Description of Artificial Sequence: Synthetic peptide
RGGRLSYSRRRFSTSTGR

SEQ ID NO: 38 - protein, 10 aa, Artificial Sequence
  Description of Artificial Sequence: Synthetic peptide
RRLSYSRRRF

SEQ ID NO: 39 - protein, 17 aa, Artificial Sequence
  Description of Artificial Sequence: Synthetic peptide
RGGRLAYLRRRWAVLGR

SEQ ID NO: 40 - protein, 11 aa, Artificial Sequence
  Description of Artificial Sequence: Synthetic peptide
YGRKKRRQRRR

SEQ ID NO: 41 - protein, 10 aa, Artificial Sequence
  Description of Artificial Sequence: Synthetic peptide
YGRKKRRQRR

SEQ ID NO: 42 - protein, 9 aa, Artificial Sequence
  Description of Artificial Sequence: Synthetic peptide
GRKKRRQRR

SEQ ID NO: 43 - protein, 13 aa, Artificial Sequence
  Description of Artificial Sequence: Synthetic peptide
GRKKRRQRRRPPQ

SEQ ID NO: 44 - protein, 11 aa, Artificial Sequence
  Description of Artificial Sequence: Synthetic peptide
GKKKKRKREKL

SEQ ID NO: 45 - protein, 8 aa, Artificial Sequence
  Description of Artificial Sequence: Synthetic peptide
SKKKKTKV

SEQ ID NO: 46 - protein, 27 aa, Artificial Sequence
  Description of Artificial Sequence: Synthetic peptide
GWTLNSAGYLLGKINLKALAALAKKIL

SEQ ID NO: 47 - protein, 21 aa, Artificial Sequence
  Description of Artificial Sequence: Synthetic peptide
AGYLLGKINLKALAALAKKIL

SEQ ID NO: 48 - protein, 12 aa, Artificial Sequence
  Description of Artificial Sequence: Synthetic peptide
PLIYLRLLRGQF

SEQ ID NO: 49 - protein, 34 aa, Artificial Sequence
  Description of Artificial Sequence: Synthetic polypeptide
DAATATRGRSAASRPTQRPRAPARSASRPRRPVQ

SEQ ID NO: 50 - protein, 16 aa, Artificial Sequence
  Description of Artificial Sequence: Synthetic peptide
  MOD_RES (1)..(16): D-amino acid
KKWKMRRNQFWIKIQR

SEQ ID NO: 51 - protein, 16 aa, Artificial Sequence
  Description of Artificial Sequence: Synthetic peptide
  MOD_RES (1)..(16): D-amino acid
KKWKMRRNQFWLKLQR

SEQ ID NO: 52 - protein, 7 aa, Artificial Sequence
  Description of Artificial Sequence: Synthetic peptide
  MOD_RES (2)..(7): Any amino acid
LXXXXXX

SEQ ID NO: 53 - protein, 22 aa, Artificial Sequence
  Description of Artificial Sequence: Synthetic peptide
  MOD_RES (4)..(4): Glu or any positively charged amino acid
  MOD_RES (5)..(5): Cys or any non-polar amino acid
  MOD_RES (6)..(6): Gln or Ala
  MOD_RES (9)..(9): Glu or any positively charged amino acid
  MOD_RES (11)..(11): Arg or any negatively charged amino acid
  MOD_RES (12)..(12): Asn or any non-polar amino acid
  MOD_RES (16)..(16): Lys or any negatively charged amino acid
  MOD_RES (21)..(21): Ser or Ala
LEGXXXGLXAXXRELXERAEXV

SEQ ID NO: 54 - protein, 22 aa, Artificial Sequence
  Description of Artificial Sequence: Synthetic peptide
LEGEGQGLEARNRELKERAESV

SEQ ID NO: 55 - protein, 22 aa, Artificial Sequence
  Description of Artificial Sequence: Synthetic peptide
LEGEAQGLEARNRELKERAESV

SEQ ID NO: 56 - protein, 22 aa, Artificial Sequence
  Description of Artificial Sequence: Synthetic peptide
LEGECQGLEARNRELKERAEAV

SEQ ID NO: 57 - protein, 22 aa, Artificial Sequence
  Description of Artificial Sequence: Synthetic peptide
LEGECQGLEARLRELKERAESV

SEQ ID NO: 58 - protein, 22 aa, Artificial Sequence
  Description of Artificial Sequence: Synthetic peptide
LEGECAGLEARNRELKERAESV

SEQ ID NO: 59 - protein, 22 aa, Artificial Sequence
  Description of Artificial Sequence: Synthetic peptide
LEGRCQGLRAENRELEERAESV

SEQ ID NO: 60 - protein, 22 aa, Artificial Sequence
  Description of Artificial Sequence: Synthetic peptide
LEGRCQGLRAELRELEERAEAV

SEQ ID NO: 61 - protein, 22 aa, Artificial Sequence
  Description of Artificial Sequence: Synthetic peptide
LEGRAQGLRAELRELEERAEAV

SEQ ID NO: 62 - protein, 22 aa, Artificial Sequence
  Description of Artificial Sequence: Synthetic peptide
LEGRLQGLRAELRELEERAEAV

SEQ ID NO: 63 - protein, 22 aa, Artificial Sequence
  Description of Artificial Sequence: Synthetic peptide
LEGRLAGLRAELRELEERAEAV

SEQ ID NO: 64 - protein, 22 aa, Artificial Sequence
  Description of Artificial Sequence: Synthetic peptide
LEGRAAGLRAELRELEERAEAV

SEQ ID NO: 65 - protein, 22 aa, Artificial Sequence
  Description of Artificial Sequence: Synthetic peptide
  MOD_RES (1)..(22): D-amino acid
VAEAREELERLEARLGQARGEL

SEQ ID NO: 66 - protein, 4 aa, Artificial Sequence
  Description of Artificial Sequence: Synthetic peptide
  MOD_RES (2)..(2): Lys or Arg
  MOD_RES (3)..(3): Any amino acid
  MOD_RES (4)..(4): Lys or Arg
KXXX

SEQ ID NO: 67 - protein, 19 aa, Artificial Sequence
  Description of Artificial Sequence: Synthetic peptide
  MOD_RES (1)..(2): Lys or Arg
  MOD_RES (3)..(14): Any amino acid
  MISC_FEATURE (3)..(14): This region may encompass 10-12 residues
  MOD_RES (15)..(19): Lys or Arg
  See specification as filed for detailed description of substitutions and preferred embodiments
XXXXXXXXXXXXXXXXXXX

SEQ ID NO: 68 - protein, 15 aa, Artificial Sequence
  Description of Artificial Sequence: Synthetic peptide
KRPAATKKAGQAKKK

SEQ ID NO: 69 - protein, 5 aa, Artificial Sequence
  Description of Artificial Sequence: Synthetic peptide
VPTLK

SEQ ID NO: 70 - protein, 5 aa, Artificial Sequence
  Description of Artificial Sequence: Synthetic peptide
KLPVM

SEQ ID NO: 71 - protein, 9 aa, Artificial Sequence
  Description of Artificial Sequence: Synthetic peptide
PAAKRVKLD

SEQ ID NO: 72 - protein, 5 aa, Artificial Sequence
  Description of Artificial Sequence: Synthetic peptide
GRGDS

SEQ ID NO: 73 - protein, 6 aa, Artificial Sequence
  Description of Artificial Sequence: Synthetic peptide
GRGDNP

SEQ ID NO: 74 - DNA, 22 bp, Artificial Sequence
  Description of Artificial Sequence: Synthetic primer
atggatgatgatatcgccgcgc

SEQ ID NO: 75 - DNA, 22 bp, Artificial Sequence
  Description of Artificial Sequence: Synthetic primer
gaagcatttgcggtggacgatg

SEQ ID NO: 76 - DNA, 15 bp, Artificial Sequence
  Description of Artificial Sequence: Synthetic primer
atggcgcacgctggg

SEQ ID NO: 77 - DNA, 21 bp, Artificial Sequence
  Description of Artificial Sequence: Synthetic primer
cttgtggcccagataggcacc

SEQ ID NO: 78 - DNA, 23 bp, Artificial Sequence
  Description of Artificial Sequence: Synthetic primer
gcccagactcacatcaccaagtg

SEQ ID NO: 79 - DNA, 25 bp, Artificial Sequence
  Description of Artificial Sequence: Synthetic primer
atgtttggcctcaaaagaaacgcgg

SEQ ID NO: 80 - DNA, 33 bp, Artificial Sequence
  Description of Artificial Sequence: Synthetic primer
tcttattagatatgccaaaccagctcctactcc

SEQ ID NO: 81 - DNA, 20 bp, Artificial Sequence
  Description of Artificial Sequence: Synthetic primer
atgtcactcctggcgaccct

SEQ ID NO: 82 - DNA, 19 bp, Artificial Sequence
  Description of Artificial Sequence: Synthetic primer
gcagctacgggtcctctgg

SEQ ID NO: 83 - DNA, 16 bp, Artificial Sequence
  Description of Artificial Sequence: Synthetic primer
atgcacctgcagcccg

SEQ ID NO: 84 - DNA, 17 bp, Artificial Sequence
  Description of Artificial Sequence: Synthetic primer
cgcgcagttgcccatgg

SEQ ID NO: 85 - DNA, 18 bp, Artificial Sequence
  Description of Artificial Sequence: Synthetic primer
atgggtgccccgacgttg

SEQ ID NO: 86 - DNA, 21 bp, Artificial Sequence
  Description of Artificial Sequence: Synthetic primer
tcaatccatggcagccagctg

SEQ ID NO: 87 - protein, 12 aa, Artificial Sequence
  Description of Artificial Sequence: Synthetic peptide
  MISC_FEATURE (1)..(12): This sequence may encompass 7-12 residues
RRRRRRRRRRRR